European Patent Application EP 4 269 599 A1, published November 1, 2023. Title: Plant cell lines producing recombinant albumin with high yield and uses thereof. Applicant: Genecell Biotech Inc.,. The sequence listing filed with the application follows.

SEQUENCE LISTING (23 sequences)

SEQ ID NO: 1 - DNA, 1837 bp, Artificial Sequence
  Canis lupus albumin
ggttaattaaggtctcaaggttctagaatcagtagtggttagcagcaactcactatcgaacacggtttcagcttacacagatatgaagtgggtgacctttatcagcctcttcttcctgttctcctcggcctactctaggggccttgttagacgcgaggcctacaagtctgagatcgcccacaggtacaacgacctcggcgaggaacatttcaggggcctcgtgctcgttgccttcagccagtacctccagcagtgcccgttcgaggatcatgtgaagctcgccaaagaggtgaccgagttcgccaaggcttgcgccgctgaggaatctggcgccaactgcgataagtccctgcacaccctcttcggcgacaagctctgcacagttgccagcctcagggacaagtacggcgacatggctgactgctgcgagaagcaagagccggatcgcaacgagtgcttcctcgcgcacaaggatgataacccgggcttcccaccactcgtggctccagaaccagatgctctctgcgccgccttccaggataacgagcaactcttcctgggcaagtacctctacgagatcgccaggcgccatccgtacttctacgctccagagctgctctactacgcccagcagtacaagggcgttttcgccgagtgctgccaagccgctgataaggctgcttgcttgggccctaagattgaggccctccgcgagaaggttctcctcagctccgcgaaagaacgcttcaagtgcgccagcctccagaagttcggcgatagagccttcaaggcctggtctgttgccaggctctctcagaggttcccgaaggccgatttcgctgagatctccaaggtggtgaccgacctcaccaaggtgcacaaagaatgctgccacggcgaccttctcgagtgcgctgatgatagagccgacctcgcgaagtacatgtgcgagaaccaggactccatctccaccaagctcaaagagtgctgcgacaagccagtgctcgagaagtctcagtgcctggccgaggttgagagggatgagcttccaggcgatctcccatctctcgccgcggatttcgtcgaggacaaagaggtctgcaagaactaccaagaggccaaggacgtgttcctcggcaccttcctgtacgagtacgctcgcaggcatccagagtactccgttagcttgctcctccgcctcgcgaaagagtacgaggctacccttgagaagtgctgcgccaccgatgatccgccaacatgctacgccaaggtgctcgacgagttcaagccgctcgtggatgagccacagaacctcgtcaagacgaactgcgagctgttcgagaagctcggcgagtacggcttccagaatgccctcctcgtgcgctacaccaagaaggccccacaggttagcaccccaactctcgttgaggtgtcacgcaagctcggcaaggtgggcacaaagtgctgcaagaagcctgagtccgagcgcatgtcttgcgccgaggatttcctctccgtggtgctcaataggctctgcgtgctccacgaaaagaccccggtttctgagcgcgtgaccaagtgctgctctgagtccctcgttaaccgcaggccatgcttctctggcctcgaggtggacgagacatacgtgccgaaagagttcaacgccgagacattcaccttccacgccgacctctgcacactcccagaggctgagaagcaggtcaagaaacagacggccctggtcgagctgctcaagcacaagccaaaggccacagacgagcagctcaagaccgtgatgggcgatttcggcgccttcgtggaaaagtgctgtgccgcc

SEQ ID NO: 2 - DNA, 1839 bp, Artificial Sequence
  Felis catus albumin
tctagaatgaagtgggtaacctttatttccctcctcctcctctttagctctgcttattccaggggcgtgactcgtcgagaagcacatcagagtgagattgctcatcggttcaatgatttgggagaagaacatttcagaggcctggtactggttgccttttctcagtatctccagcagtgtccatttgaagatcatgtaaaattagtgaatgaagtaactgagttcgcaaaaggatgtgtggctgaccagtcagcagccaactgtgaaaagtcacttcacgaactcttaggagataaactgtgtacagttgcctctcttcgcgacaagtatggtgagatggctgattgctgtgagaaaaaagaacctgagagaaacgaatgcttcctgcagcacaaagatgacaatcccggcttcggtcagctggtgaccccagaggctgatgccatgtgcactgccttccacgaaaatgaacagaggttcctgggcaaatacttatatgaaattgccagaagacatccttacttttatgccccagaactcctttactatgccgaagaatacaaaggagtttttacagaatgctgcgaagctgcagataaagctgcctgcctgacaccaaaggttgatgctttgagagaaaaagtactggcttcatccgccaaagagagactcaagtgtgccagcctccagaaattcggagaaagagctttcaaagcatggtcagtagctcgtctgagccagaaatttcccaaggctgaatttgcagagatttccaagttagtgacagatcttgccaaaatccacaaggaatgctgccatggtgacctgcttgaatgtgcagatgacagggcggaccttgccaagtatatatgtgaaaatcaagattcaatctccactaagctgaaggaatgctgtggtaagcctgtgttggaaaaatcccattgcatcagcgaggtggaaagagatgagttgcctgctgacctgcccccgttagctgttgattttgttgaagataaggaagtttgcaagaactatcaggaggcaaaggatgtgttcctgggcacgtttttgtatgaatactcaagaaggcaccctgaatactctgtctcattgctactgagacttgccaaggaatatgaagccaccctagagaagtgctgtgccactgatgatcctcctgcttgctatgcccatgtgtttgatgaatttaaacctcttgtggaagagcctcacaatttagtcaaaacaaactgtgaactttttgaaaaacttggagaatatggcttccaaaatgcgctcttagttcgttacaccaagaaagtacctcaagtgtcaactccaactctcgtggaggtctcaagaagcctaggaaaagtgggcagcaagtgttgtacgcatcctgaagcagaaagactgtcctgtgctgaagactatctgtccgtggtcctgaaccggttgtgtgtgttgcatgagaagacccctgtgagcgagagagttaccaaatgctgcacagagtccttggtgaacagacgaccatgcttttctgctctgcaagtcgatgaaacatatgttcccaaagaatttagtgctgaaacattcaccttccatgcagatttatgcacacttcctgaggctgagaaacaaatcaagaaacaatctgcacttgttgagctgttgaaacacaagcccaaggcaacagaggaacaactgaaaactgtcatgggggattttggaagctttgtagacaagtgctgcgcagctgaagacaaggaggcctgctttgctgaggagggtccaaagcttgttgctgcagctcaagctgccttagcctaaggtacc

SEQ ID NO: 3 - DNA, 20 bp, Artificial Sequence
  forward primer F1
gcaagtacctctacgagatc

SEQ ID NO: 4 - DNA, 20 bp, Artificial Sequence
  reverse primer R1
tgcgctcggtctcaggcttc

SEQ ID NO: 5 - DNA, 20 bp, Artificial Sequence
  forward primer F2
cagagcgcaacgagtgcttc

SEQ ID NO: 6 - DNA, 20 bp, Artificial Sequence
  reverse primer R2
tctgtacagcacttcgtcac

SEQ ID NO: 7 - DNA, 1940 bp, Artificial Sequence
  RAmy3A-Canis lupus albumin
ggttaattaaggtctcaaggttctagaatcagtagtggttagcagcaactcactatcgaacacggtttcagcttacacagatatgggcaagcaaatggctgctctctgcggcttcctcctcgtggctctcttgtggctcacaccagatgttgcccatgccgaggcctacaagtctgagatcgcccacaggtacaacgacctcggcgaggaacatttcaggggcctcgtgctcgttgccttcagccagtacctccagcagtgcccgttcgaggatcatgtgaagctcgccaaagaggtgaccgagttcgccaaggcttgcgccgctgaggaatctggcgccaactgcgataagtccctgcacaccctcttcggcgacaagctttgcacagttgccagcctcagggacaagtacggcgacatggctgactgctgcgagaagcaagagccggatcgcaacgagtgcttcctcgcgcacaaggatgataacccgggcttcccaccacttgtggccccagaaccagatgctctttgcgccgccttccaggacaacgagcaactcttcctgggcaagtacctctacgagatcgccaggcgccatccgtacttctacgctccagagctgctctactacgcccagcagtacaagggcgttttcgccgagtgctgccaagccgctgataaggctgcttgcttgggccctaagattgaggccctccgcgagaaggttctcctcagctccgcgaaagaacgcttcaagtgcgccagcctccagaagttcggcgatagagccttcaaggcctggtctgttgccaggctctctcagaggttcccgaaggccgatttcgctgagatctccaaggtggtgaccgacctcaccaaggtgcacaaagaatgctgccacggcgacctgcttgagtgcgctgatgatagagccgacctcgcgaagtacatgtgcgagaaccaggactccatctccaccaagctcaaagagtgctgcgacaagccagtgcttgagaagtctcagtgcctggcggaggtcgagagggatgaacttccaggcgatctcccatctctcgccgccgacttcgttgaggacaaagaggtctgcaagaactaccaagaggccaaggacgtgttcctcggcaccttcctgtacgagtacgctcgcaggcatccagagtactccgttagcttgctcctccgcctcgcgaaagagtacgaggcgacattggagaagtgctgcgccaccgatgatccgccaacatgctacgccaaggtgctcgacgagttcaagccgctcgttgacgagccacagaacctcgtcaagacgaactgcgagctgttcgagaagctcggcgagtacggcttccagaatgccctcctcgtccgctacaccaagaaggccccacaggttagcaccccaactctcgttgaggtgtcacgcaagctcggcaaggtgggcacaaagtgctgcaagaagcctgagtccgagcgcatgtcttgcgccgaggatttcctctccgtggtgctcaataggctctgcgtgctccacgaaaagaccccggtttctgagcgcgtgaccaagtgctgctctgagtccctcgttaaccgcaggccatgcttctctggccttgaggtggacgagacatacgtgccgaaagagttcaacgccgagacattcaccttccacgccgacctctgcacactcccagaggctgagaagcaggtcaagaaacagaccgcgctggtcgagctgctcaagcacaagccaaaggccacagacgagcagctcaagaccgtgatgggcgatttcggcgccttcgtggaaaagtgctgtgccgcggagaacaaagagggatgcttcagcgaagagggcccgaagttggttgctgccgctcaagctgctctcgtgtgataggtaccgctttgagaccctcgag

SEQ ID NO: 8 - DNA, 1925 bp, Artificial Sequence
  VspA-Canis lupus albumin
ggttaattaaggtctcaaggttctagaatcagtagtggttagcagcaactcactatcgaacacggtttcagcttacacagatatgaagatggtggtgctcgtgttcttcgtggccaccattctcgtggcctggcaatgccacgccgaggcctacaagtctgagatcgcccacaggtacaacgacctcggcgaggaacatttcaggggcctcgtgctcgttgccttcagccagtacctccagcagtgcccgttcgaggatcatgtgaagctcgccaaagaggtgaccgagttcgccaaggcttgcgccgctgaggaatctggcgccaactgcgataagtccctgcacaccctcttcggcgacaagctttgcacagttgccagcctcagggacaagtacggcgacatggctgactgctgcgagaagcaagagccggatcgcaacgagtgcttcctcgcgcacaaggatgataacccgggcttcccaccacttgtggccccagaaccagatgctctttgcgccgccttccaggacaacgagcaactcttcctgggcaagtacctctacgagatcgccaggcgccatccgtacttctacgctccagagctgctctactacgcccagcagtacaagggcgttttcgccgagtgctgccaagccgctgataaggctgcttgcttgggccctaagattgaggccctccgcgagaaggttctcctcagctccgcgaaagaacgcttcaagtgcgccagcctccagaagttcggcgatagagccttcaaggcctggtctgttgccaggctctctcagaggttcccgaaggccgatttcgctgagatctccaaggtggtgaccgacctcaccaaggtgcacaaagaatgctgccacggcgacctgcttgagtgcgctgatgatagagccgacctcgcgaagtacatgtgcgagaaccaggactccatctccaccaagctcaaagagtgctgcgacaagccagtgcttgagaagtctcagtgcctggcggaggtcgagagggatgaacttccaggcgatctcccatctctcgccgccgacttcgttgaggacaaagaggtctgcaagaactaccaagaggccaaggacgtgttcctcggcaccttcctgtacgagtacgctcgcaggcatccagagtactccgttagcttgctcctccgcctcgcgaaagagtacgaggcgacattggagaagtgctgcgccaccgatgatccgccaacatgctacgccaaggtgctcgacgagttcaagccgctcgttgacgagccacagaacctcgtcaagacgaactgcgagctgttcgagaagctcggcgagtacggcttccagaatgccctcctcgtccgctacaccaagaaggccccacaggttagcaccccaactctcgttgaggtgtcacgcaagctcggcaaggtgggcacaaagtgctgcaagaagcctgagtccgagcgcatgtcttgcgccgaggatttcctctccgtggtgctcaataggctctgcgtgctccacgaaaagaccccggtttctgagcgcgtgaccaagtgctgctctgagtccctcgttaaccgcaggccatgcttctctggccttgaggtggacgagacatacgtgccgaaagagttcaacgccgagacattcaccttccacgccgacctctgcacactcccagaggctgagaagcaggtcaagaaacagaccgcgctggtcgagctgctcaagcacaagccaaaggccacagacgagcagctcaagaccgtgatgggcgatttcggcgccttcgtggaaaagtgctgtgccgcggagaacaaagagggatgcttcagcgaagagggcccgaagttggttgctgccgctcaagctgctctcgtgtgataggtaccgctttgagaccctcgag

SEQ ID NO: 9 - DNA, 1940 bp, Artificial Sequence
  RAmy3A-Felis catus albumin
ggttaattaaggtctcaaggttctagaatcagtagtggttagcagcaactcactatcgaacacggtttcagcttacacagatatgggcaagcaaatggctgctctctgcggcttcctcctcgtggctctcttgtggctcacaccagatgtggcccatgccgaggctcatcagtctgagatcgcccacaggttcaacgacctcggcgaggaacatttcaggggcctcgtgctcgttgccttcagccagtacctccagcagtgcccgttcgaggatcacgtgaagctcgtgaacgaggtgaccgagttcgccaagggatgcgtggcagatcaatccgccgccaactgcgagaagtccctccatgaactcctcggcgacaagctttgcacagttgccagcctcagggacaagtacggcgagatggctgactgctgcgaaaagaaagagccagagcgcaacgagtgcttcctccagcacaaggacgacaacccaggcttcggccaactcgttacaccagaggccgatgccatgtgcaccgccttccatgagaatgagcaacgcttcctcggcaagtacctctacgagatcgctcgcaggcacccgtacttctacgctccagagcttctctactacgccgaagagtacaagggcgtgttcaccgagtgctgcgaggccgccgataaggctgcttgcctcacaccaaaagtggacgccctccgcgagaaggttttggcctcttccgccaaagaacgcctcaagtgcgccagcctccaaaagtttggcgagagggccttcaaggcctggtctgttgctaggctctcccagaagttcccgaaggctgagttcgccgagatctccaagctcgtcaccgacctcgccaagatccacaaagaatgctgccacggcgacctgcttgagtgcgctgatgatagagccgacctggcgaagtacatctgcgagaaccaggactccatctccaccaagctcaaagagtgttgcggcaagccggtgctcgaaaagtcccactgcatctccgaggtcgagagggatgagcttccagcggatctcccaccactcgccgtggatttcgtcgaggacaaagaggtgtgcaagaactaccaagaggcgaaggacgtgttcctgggcaccttcctgtacgagtactcccgcaggcatccagagtactccgttagcttgctcctccgcctcgccaaagagtacgaggcgacacttgagaagtgctgcgccaccgatgatccgccagcctgctacgcccatgtgttcgatgagttcaagccgctggtcgaggaaccgcacaacctcgtcaagacgaactgcgagctgttcgagaagctcggcgagtacggcttccagaatgccctcctcgtccgctacaccaagaaggtcccacaggtcagcaccccgacactcgttgaggtgtcaagatctctcggcaaggtgggctccaagtgctgcacacatccagaggctgagagactctcctgcgccgaggattacctctccgtggtgctcaataggctctgcgtgctccacgaaaagaccccggtttctgagcgcgtgacgaagtgctgtacagagtccctcgtgaaccgcaggccatgcttctctgccctccaagtggacgagacatacgtgccgaaagagttctccgccgagacattcaccttccacgccgacctctgcactttgcctgaggccgagaagcagatcaagaaacagagcgccctcgtcgagctgctcaagcacaagccaaaggccaccgaggaacagctcaagaccgtgatgggcgacttcggctccttcgtggataagtgctgtgccgcggaggacaaagaagcctgctttgctgaagagggcccgaagctcgttgctgccgctcaagctgccctcgcctgataggtaccgctttgagaccctcgag

SEQ ID NO: 10 - DNA, 1925 bp, Artificial Sequence
  VspA-Felis catus albumin
ggttaattaaggtctcaaggttctagaatcagtagtggttagcagcaactcactatcgaacacggtttcagcttacacagatatgaagatggtggtgctcgtgttcttcgtggccaccattctcgtggcctggcaatgccacgccgaggctcatcagtctgagatcgcccacaggttcaacgacctcggcgaggaacatttcaggggcctcgtgctcgttgccttcagccagtacctccagcagtgcccgttcgaggatcacgtgaagctcgtgaacgaggtgaccgagttcgccaagggatgcgtggcagatcaatccgccgccaactgcgagaagtccctccatgaactcctcggcgacaagctttgcacagttgccagcctcagggacaagtacggcgagatggctgactgctgcgaaaagaaagagccagagcgcaacgagtgcttcctccagcacaaggacgacaacccaggcttcggccaactcgttacaccagaggccgatgccatgtgcaccgccttccatgagaatgagcaacgcttcctcggcaagtacctctacgagatcgctcgcaggcacccgtacttctacgctccagagcttctctactacgccgaagagtacaagggcgtgttcaccgagtgctgcgaggccgccgataaggctgcttgcctcacaccaaaagtggacgccctccgcgagaaggttttggcctcttccgccaaagaacgcctcaagtgcgccagcctccaaaagtttggcgagagggccttcaaggcctggtctgttgctaggctctcccagaagttcccgaaggctgagttcgccgagatctccaagctcgtcaccgacctcgccaagatccacaaagaatgctgccacggcgacctgcttgagtgcgctgatgatagagccgacctggcgaagtacatctgcgagaaccaggactccatctccaccaagctcaaagagtgttgcggcaagccggtgctcgaaaagtcccactgcatctccgaggtcgagagggatgagcttccagcggatctcccaccactcgccgtggatttcgtcgaggacaaagaggtgtgcaagaactaccaagaggcgaaggacgtgttcctgggcaccttcctgtacgagtactcccgcaggcatccagagtactccgttagcttgctcctccgcctcgccaaagagtacgaggcgacacttgagaagtgctgcgccaccgatgatccgccagcctgctacgcccatgtgttcgatgagttcaagccgctggtcgaggaaccgcacaacctcgtcaagacgaactgcgagctgttcgagaagctcggcgagtacggcttccagaatgccctcctcgtccgctacaccaagaaggtcccacaggtcagcaccccgacactcgttgaggtgtcaagatctctcggcaaggtgggctccaagtgctgcacacatccagaggctgagagactctcctgcgccgaggattacctctccgtggtgctcaataggctctgcgtgctccacgaaaagaccccggtttctgagcgcgtgacgaagtgctgtacagagtccctcgtgaaccgcaggccatgcttctctgccctccaagtggacgagacatacgtgccgaaagagttctccgccgagacattcaccttccacgccgacctctgcactttgcctgaggccgagaagcagatcaagaaacagagcgccctcgtcgagctgctcaagcacaagccaaaggccaccgaggaacagctcaagaccgtgatgggcgacttcggctccttcgtggataagtgctgtgccgcggaggacaaagaagcctgctttgctgaagagggcccgaagctcgttgctgccgctcaagctgccctcgcctgataggtaccgctttgagaccctcgag

SEQ ID NO: 11 - protein, 26 aa, Oryza sativa
MGKQMAALCGFLLVALLWLTPDVAHA

SEQ ID NO: 12 - protein, 21 aa, Glycine max
MKMVVLVFFVATILVAWQCHA

SEQ ID NO: 13 - protein, 27 aa, Nicotiana tabacum
MATQRRANPSSLHLITVFSLLVAVVSA

SEQ ID NO: 14 - protein, 26 aa, Malus domestica
MALKTQLLWSFVVVFVVSFSTTSCSG

SEQ ID NO: 15 - protein, 24 aa, Hordeum vulgare
MGKNGSLCCFSLLLLLLLAGLASG

SEQ ID NO: 16 - protein, 24 aa, Hordeum vulgare
MANKHLSLSLFLVLLGLSASLASG

SEQ ID NO: 17 - protein, 25 aa, Oryza sativa
MKNTSSLCLLLLVVLCSLTCNSGQA

SEQ ID NO: 18 - protein, 24 aa, Oryza sativa
MASINRPIVFFTVCLFLLCNGSLA

SEQ ID NO: 19 - protein, 26 aa, Nicotiana benthamiana
MGKMASLFATLLVVLVSLSLASESSA

SEQ ID NO: 20 - protein, 23 aa, Nicotiana benthamiana
MLPFSLLVSTLLLFLVISHSCRA

SEQ ID NO: 21 - protein, 24 aa, Medicago truncatula
MAKNVSIFGLLFSLLALVPSQIFA

SEQ ID NO: 22 - protein, 22 aa, Oryza sativa
MGTRLLALAPWLLLLLLQLAGA

SEQ ID NO: 23 - protein, 25 aa, Oryza sativa
MAALSQLVLVTAFLAAALLPLGMAA